European Patent Application EP 4 257 607 A1, published October 11, 2023. Title: DEVELOPMENT AND APPLICATION OF T-CELL ENGAGER THERAPEUTIC AGENT. Applicant: KEYMED BIOSCIENCES CO., LTD. The sequence listing filed with the application follows.

SEQUENCE LISTING (185 sequences)

SEQ ID NO: 1 - protein, 290 aa, Homo sapiens
MLQMAGQCSQNEYFDSLLHACIPCQLRCSSNTPPLTCQRYCNASVTNSVKGTNASGAEPRGPTIKPCPPCKCPAPNLLGGPSVFIFPPKIKDVLMISLSPIVTCVVVDVSEDDPDVQISWFVNNVEVHTAQTQTHREDYNSTLRVVSALPIQHQDWMSGKEFKCKVNNKDLPAPIERTISKPKGSVRAPQVYVLPPPEEEMTKKQVTLTCMVTDFMPEDIYVEWTNNGKTELNYKNTEPVLDSDGSYFMYSKLRVEKKNWVERNSYSCSVVHEGLHNHHTTKSFSRTPGK

SEQ ID NO: 2 - protein, 290 aa, Macaca fascicularis
MLQMARQCSQNEYFDSLLHDCKPCQLRCSSTPPLTCQRYCNASMTNSVKGMNAASGAEPRGPTIKPCPPCKCPAPNLLGGPSVFIFPPKIKDVLMISLSPIVTCVVVDVSEDDPDVQISWFVNNVEVHTAQTQTHREDYNSTLRVVSALPIQHQDWMSGKEFKCKVNNKDLPAPIERTISKPKGSVRAPQVYVLPPPEEEMTKKQVTLTCMVTDFMPEDIYVEWTNNGKTELNYKNTEPVLDSDGSYFMYSKLRVEKKNWVERNSYSCSVVHEGLHNHHTTKSFSRTPGK

SEQ ID NO: 3 - protein, 304 aa, Homo sapiens
MLQMAGQCSQNEYFDSLLHACIPCQLRCSSNTPPLTCQRYCNASVTNSVKGTNASGGGGSDKTHTCPPCPAPEAAGGPSVFLFPPKPKDTLMISRTPEVTCVVVDVSHEDPEVKFNWYVDGVEVHNAKTKPREEQYNSTYRVVSVLTVLHQDWLNGKEYKCKVSNKALPASIEKTISKAKGQPREPQVYTLPPCRDELTKNQVSLWCLVKGFYPSDIAVEWESNGQPENNYKTTPPVLDSDGSFFLYSKLTVDKSRWQQGNVFSCSVMHEALHNHYTQKSLSLSPGKGSGLNDIFEAQKIEWHE

SEQ ID NO: 4 - protein, 303 aa, Macaca fascicularis
MLQMARQCSQNEYFDSLLHDCKPCQLRCSSTPPLTCQRYCNASMTNSVKGMNASGGGGSDKTHTCPPCPAPEAAGGPSVFLFPPKPKDTLMISRTPEVTCVVVDVSHEDPEVKFNWYVDGVEVHNAKTKPREEQYNSTYRVVSVLTVLHQDWLNGKEYKCKVSNKALPASIEKTISKAKGQPREPQVYTLPPCRDELTKNQVSLWCLVKGFYPSDIAVEWESNGQPENNYKTTPPVLDSDGSFFLYSKLTVDKSRWQQGNVFSCSVMHEALHNHYTQKSLSLSPGKGSGLNDIFEAQKIEWHE

SEQ ID NO: 5 - protein, 227 aa, Homo sapiens
DKTHTCPPCPAPEAAGGPSVFLFPPKPKDTLMISRTPEVTCVVVDVSHEDPEVKFNWYVDGVEVHNAKTKPREEQYNSTYRVVSVLTVLHQDWLNGKEYKCKVSNKALPASIEKTISKAKGQPREPQVCTLPPSRDELTKNQVSLSCAVKGFYPSDIAVEWESNGQPENNYKTTPPVLDSDGSFFLVSKLTVDKSRWQQGNVFSCSVMHEALHNHYTQKSLSLSPGK

SEQ ID NO: 6 - protein, 306 aa, Homo sapiens
QSIKGNHLVKVYDYQEDGSVLLTCDAEAKNITWFKDGKMIGFLTEDKKKWNLGSNAKDPRGMYQCKGSQNKSKPLQVYYRMCQNCIELNAPEAAGGPSVFLFPPKPKDTLMISRTPEVTCVVVDVSHEDPEVKFNWYVDGVEVHNAKTKPREEQYNSTYRVVSVLTVLHQDWLNGKEYKCKVSNKALPASIEKTISKAKGQPREPQVCTLPPSRDELTKNQVSLSCAVKGFYPSDIAVEWESNGQPENNYKTTPPVLDSDGSFFLVSKLTVDKSRWQQGNVFSCSVMHEALHNHYTQKSLSLSPGK

SEQ ID NO: 7 - protein, 306 aa, Homo sapiens; identical to SEQ ID NO: 6

SEQ ID NO: 8 - protein, 305 aa, Macaca fascicularis
QSFEENRKLNVYNQEDGSVLLTCHVKNTNITWFKEGKMIDILTAHKNKWNLGSNTKDPRGVYQCKGSKDKSKTLQVYYRMCQNCIELNAPEAAGGPSVFLFPPKPKDTLMISRTPEVTCVVVDVSHEDPEVKFNWYVDGVEVHNAKTKPREEQYNSTYRVVSVLTVLHQDWLNGKEYKCKVSNKALPASIEKTISKAKGQPREPQVCTLPPSRDELTKNQVSLSCAVKGFYPSDIAVEWESNGQPENNYKTTPPVLDSDGSFFLVSKLTVDKSRWQQGNVFSCSVMHEALHNHYTQKSLSLSPGK

SEQ ID NO: 9 - protein, 330 aa, Macaca fascicularis
QDGNEEMGSITQTPYQVSISGTTVILTCSQHLGSEAQWQHNGKNKEDSGDRLFLPEFSEMEQSGYYVCYPRGSNPEDASHHLYLKARVCENCMEMDAPEAAGGPSVFLFPPKPKDTLMISRTPEVTCVVVDVSHEDPEVKFNWYVDGVEVHNAKTKPREEQYNSTYRVVSVLTVLHQDWLNGKEYKCKVSNKALPASIEKTISKAKGQPREPQVYTLPPCRDELTKNQVSLWCLVKGFYPSDIAVEWESNGQPENNYKTTPPVLDSDGSFFLYSKLTVDKSRWQQGNVFSCSVMHEALHNHYTQKSLSLSPGKGSGLNDIFEAQKIEWHE

SEQ ID NO: 10 - protein, 122 aa, Homo sapiens
EIQLVQSGPELKKPGETVKISCKASGYIFTNFGMNWVRQAPGKALKWMGWINTYTGEQIYADDFKGRFAFSLETSASTAYLQINNLKNEDTATYFCARGEIYYGYDVGFVYWGQGTLVTVSA

SEQ ID NO: 11 - DNA, 366 bp, Homo sapiens
gagatccagttggtgcagtctggacctgagctgaagaagcctggagagacagtcaagatctcctgcaaggcttctgggtatatcttcacaaactttggaatgaactgggtgaggcaggctccaggaaaggctttaaagtggatgggctggataaacacctacactggagaacaaatatatgctgatgacttcaagggacggtttgccttctctttggaaacctctgccagcactgcctatttgcagatcaacaacctcaaaaatgaggacacggctacatatttctgtgcaagaggggagatctactatggttacgacgtgggctttgtttactggggccaagggactctggtcactgtctctgca

SEQ ID NO: 12 - protein, 6 aa, Mus musculus
TNFGMN

SEQ ID NO: 13 - protein, 17 aa, Mus musculus
WINTYTGEQIYADDFKG

SEQ ID NO: 14 - protein, 13 aa, Mus musculus
GEIYYGYDVGFVY

SEQ ID NO: 15 - protein, 111 aa, Mus musculus
DIVLTQSPASLTVSLGQRATISCRASKSVSTSGYSYMHWYQQKPGQPPKLLIYLASDLESGVSARFSGSGSGTDFTLNIHPVEEEDAATYYCQHSRELPWTFGGGTKLEIK

SEQ ID NO: 16 - DNA, 333 bp, Mus musculus
gatattgtgctaactcagtctcctgcttccttaactgtatctctggggcagagggccaccatctcatgcagggccagcaaaagtgtcagtacatctggctatagttatatgcactggtaccaacagaaaccaggacagccacccaaactcctcatctatcttgcatccgacctagaatctggggtctctgccaggttcagtggcagtgggtctgggacagacttcaccctcaacatccatcctgtggaggaggaggatgctgcaacctattactgtcaacacagtagggaacttccgtggacgttcggtggaggcaccaagctggaaataaaa

SEQ ID NO: 17 - protein, 15 aa, Mus musculus
RASKSVSTSGYSYMH

SEQ ID NO: 18 - protein, 7 aa, Mus musculus
LASDLES

SEQ ID NO: 19 - protein, 9 aa, Mus musculus
QHSRELPWT

SEQ ID NO: 20 - protein, 111 aa, Mus musculus
DIVLTQSPASLAISLGQRATISCRASKSVTTSGYSYIHWYQQKPGQPPKLLIYLASDLEAGVPARFSGSGSGTDFTLNIHPVEEEDAATYYCQHSRELPWTFGGGTKLELK

SEQ ID NO: 21 - DNA, 333 bp, Mus musculus
gacattgtgctaacacagtctcctgcttccttagctatatctctggggcagagggccaccatctcatgcagggccagcaaaagtgtcactacatctggctatagttatatacactggtaccaacagaaaccaggacagccacccaaactcctcatctatcttgcatccgacctagaagctggggtccctgccaggttcagtggcagtgggtctgggacagacttcaccctcaacatccatcctgtggaggaagaggatgctgcaacctattactgtcagcacagtagggagcttccgtggacgttcggtggaggcaccaagctggagctgaaa

SEQ ID NO: 22 - protein, 15 aa, Mus musculus
RASKSVTTSGYSYIH

SEQ ID NO: 23 - protein, 7 aa, Mus musculus
LASDLEA

SEQ ID NO: 24 - protein, 118 aa, Mus musculus
QVQLQQSGPELVKPGASVNLSCKASGYTFTNYVIHWVKQKPGQGLEWIGYTIPYTDVTKYNEKFKAKATLTSDKSSSTAFMELSSLTSEDSAVYYCARYDFDGYFDYWGQGTTLTVSS

SEQ ID NO: 25 - DNA, 354 bp, Mus musculus
caggtccagctgcaacagtctggacctgagctggtgaagcctggggcttcagtgaatttgtcctgcaaggcttctggatacacattcactaattatgttatacactgggtaaagcagaagcctgggcagggccttgagtggattggatatactatcccttacactgatgttactaagtacaatgagaaattcaaagccaaggccacactgacttcagacaaatcctccagcacagccttcatggagctcagcagcctgacctctgaggactctgcggtctattactgtgcaagatatgatttcgacggctactttgactactggggccaaggcaccactctcacagtctcctca

SEQ ID NO: 26 - protein, 6 aa, Mus musculus
TNYVIH

SEQ ID NO: 27 - protein, 17 aa, Mus musculus
YTIPYTDVTKYNEKFKA

SEQ ID NO: 28 - protein, 9 aa, Mus musculus
YDFDGYFDY

SEQ ID NO: 29 - protein, 112 aa, Mus musculus
DIVMTQAAFSNPVTLGTSASISCRSSKSLLHSNGITYLYWYLQKPGQSPQLLIYQMSNLASGVPDRFSSSGSGTDFTLRISRVEAEDVGVYYCAQNLELPWTFGGGTKLELK

SEQ ID NO: 30 - DNA, 336 bp, Mus musculus
gatattgtgatgactcaggctgcattctccaatccagtcactcttggaacatcagcttccatctcctgcaggtctagtaagagtctcctacatagtaatggcatcacttatttgtattggtatctgcagaagccaggccagtctcctcagctcctgatttatcagatgtccaaccttgcctcaggagtcccagacaggttcagtagcagtgggtcaggaactgatttcacactgagaatcagcagagtggaggctgaggatgtgggtgtttattactgtgctcaaaatctagaacttccgtggacgttcggtggaggcaccaagctggagctgaaa

SEQ ID NO: 31 - protein, 16 aa, Mus musculus
RSSKSLLHSNGITYLY

SEQ ID NO: 32 - protein, 7 aa, Mus musculus
QMSNLAS

SEQ ID NO: 33 - protein, 9 aa, Mus musculus
AQNLELPWT

SEQ ID NO: 34 - protein, 122 aa, Mus musculus
EVQLQQSGPELKKPGETVKISCKASGYTFTNFGMNWVRQTPGKALKWMGWINTYTGDLIYGDDFKGRFAFSLETSASTAYLQINNLKNEDTATYFCARGEIYYGYDVGFAYWGQGTLVTVSA

SEQ ID NO: 35 - DNA, 366 bp, Mus musculus
gaggtccagctgcagcagtctggacctgagctgaagaagcctggagagacagtcaagatctcctgcaaggcttctgggtataccttcacaaactttggaatgaactgggtgaggcagactccaggaaaggctttaaagtggatgggctggataaacacctacactggagacttaatatatggtgatgactttaagggacggtttgccttctctttggaaacctctgccagcactgcctatttacagatcaacaacctcaaaaatgaggacacggctacatatttctgtgcaagaggggagatctactatggttacgacgtggggtttgcttactggggccaagggactctggtcactgtctctgca

SEQ ID NO: 36 - protein, 17 aa, Mus musculus
WINTYTGDLIYGDDFKG

SEQ ID NO: 37 - protein, 13 aa, Mus musculus
GEIYYGYDVGFAY

SEQ ID NO: 38 - protein, 111 aa, Mus musculus
DIVLTQSPASLAVSLGQRATISCRASKSVSTSGYSYMHWYQQKPGQPPKLLIYLASNLESGVPARFSGSGSGTDFTLNIHPVEEEDAATYYCQHSRELPWTFGGGTKLEIK

SEQ ID NO: 39 - DNA, 333 bp, Mus musculus
gacattgtgctgacacagtctcctgcttccttagctgtatctctggggcagagggccaccatctcatgcagggccagcaaaagtgtcagtacatctggctatagttatatgcactggtaccaacagaaaccaggacagccacccaaactcctcatctatcttgcatccaacctagaatctggggtccctgccaggttcagtggtagtgggtctgggacagacttcaccctcaacatccatcctgtggaggaggaggatgctgcaacctattactgtcagcacagtagggagcttccgtggacgttcggtggaggcaccaagctggaaatcaaa

SEQ ID NO: 40 - protein, 7 aa, Mus musculus
LASNLES

SEQ ID NO: 41 - protein, 122 aa, Mus musculus
EIQLVQSGPELKKPGETVKISCKASGYIFTNFGMNWVRQTPGKALKWMGWINTYTGETIYADDFKGLFAFSLEVPASTAYLQINNLKNEDTATYFCARGEIYYGFDVGFAYWGQGTLVTVSA

SEQ ID NO: 42 - DNA, 366 bp, Mus musculus
gagatccagttggtgcagtctggacctgagctgaagaagcctggagagacagtcaagatctcctgcaaggcttctgggtatattttcacaaactttggaatgaactgggtgaggcagactccaggaaaggctttaaagtggatgggctggataaacacctacactggagaaacaatatatgctgatgacttcaagggactatttgccttctctttggaagtgcctgccagcactgcctatttgcagatcaacaacctcaaaaatgaggacacggctacatatttctgtgcaagaggggagatctactatggtttcgacgtgggatttgcttactggggccaagggactctggtcactgtctctgca

SEQ ID NO: 43 - protein, 17 aa, Mus musculus
WINTYTGETIYADDFKG

SEQ ID NO: 44 - protein, 13 aa, Mus musculus
GEIYYGFDVGFAY

SEQ ID NO: 45 - protein, 111 aa, Mus musculus
DIVLTQSPASLTVSLGQRATISCRASKSVSTSGYSYIHWYQQKPGQPPKLLIYLASDLESGVPARFSGSGSGTDFTLNIHPVEEEDAATYYCQHSRELPWTFGGGTKLELK

SEQ ID NO: 46 - DNA, 333 bp, Mus musculus
gacattgtgctaacacagtctcctgcttccttaactgtatctctggggcagagggccaccatctcatgcagggccagcaaaagtgtcagtacatctggctatagttatatacactggtaccaacagaaaccaggacagccacccaaactcctcatctatcttgcatccgacctagaatctggggtccctgccaggttcagtggcagtgggtctgggacagacttcaccctcaacatccatcctgtggaggaggaggatgctgcaacctattactgtcaacacagtagggaacttccgtggacgttcggtggaggcaccaagctggagctgaaa

SEQ ID NO: 47 - protein, 15 aa, Mus musculus
RASKSVSTSGYSYIH

SEQ ID NO: 48 - protein, 122 aa, Mus musculus
EIQLVQSGPELKKPGETVKISCTASGYTFTNFGMNWVRQAPGKALRWMGWINTYTGDQIYADDFKGRFAFSLETSASTAYLQINNLKNEDTATYFCARGEIYYGYDVGFVYWGQGTLVTVSA

SEQ ID NO: 49 - DNA, 366 bp, Mus musculus
gagatccagttggtgcagtctggacctgagctgaagaagcctggagagacagtcaagatctcctgcacggcttctgggtataccttcacaaactttggaatgaactgggtgaggcaggctccaggaaaggctttaaggtggatgggctggataaacacctacactggagaccaaatatatgctgatgacttcaagggacggtttgccttctctttggaaacctctgccagcactgcctatttgcagatcaacaacctcaaaaatgaggacacggctacatatttctgtgcaagaggggagatctactatggttacgacgtgggctttgtttattggggccaagggactctggtcactgtctctgca

SEQ ID NO: 50 - protein, 17 aa, Mus musculus
WINTYTGDQIYADDFKG

SEQ ID NO: 51 - protein, 111 aa, Mus musculus; identical to SEQ ID NO: 38

SEQ ID NO: 52 - DNA, 333 bp, Mus musculus
gacattgtgctaacacagtctcctgcttccttagctgtatctctggggcagagggccaccatctcatgcagggccagcaaaagtgtcagtacatctggctatagttatatgcactggtaccaacagaaaccaggacagccacccaaactcctcatctatcttgcatccaacctagaatctggggtccctgccaggttcagtggcagtgggtctgggacagacttcaccctcaacatccatcctgtggaggaggaggatgctgcaacctattactgtcagcacagtagggagcttccgtggacgttcggtggaggcaccaagctggaaataaaa

SEQ ID NO: 53 - protein, 113 aa, Mus musculus
EVQLQQSGTVLTRPGASVKLSCKASGYSFSSYWMHWLKQRPGQGLEWIGAIYPGNSRTTYNQKFKGEAKLTADTSASTAYMDLSSLTNADSAVYFCTREETYWGQGTLVTVSA

SEQ ID NO: 54 - DNA, 339 bp, Mus musculus
gaggttcagctccagcagtctgggactgtgctgacaaggcctggggcttccgtgaagttgtcctgcaaggcttctggctacagcttttccagctactggatgcactggctaaaacagaggcctggacagggtctagaatggattggtgctatttatcctggaaatagtcgtactacctacaaccagaagttcaagggcgaggccaaactgactgcggacacttccgccagcactgcctacatggacctcagcagcctgacaaatgccgactctgcggtctatttctgtacaagagaggagacttactggggccaagggactctggtcactgtctctgca

SEQ ID NO: 55 - protein, 6 aa, Mus musculus
SSYWMH

SEQ ID NO: 56 - protein, 17 aa, Mus musculus
AIYPGNSRTTYNQKFKG

SEQ ID NO: 57 - protein, 6 aa, Mus musculus
TREETY

SEQ ID NO: 58 - protein, 112 aa, Mus musculus
DVVMTQTPLSLSVTIGQPASISCKSSQGLLDSYGVTYLNWLFQRPGQPPKRLIYLVSELDSGVPDRFTGSGSGTDFTLRISRVEAEDLGIYYCWQGSHFPLTFGAGTKLELK

SEQ ID NO: 59 - DNA, 336 bp, Mus musculus
gatgttgtgatgacccagactccactctctttgtcggttaccattggacaaccagcctccatctcttgcaagtcaagtcagggcctcttagatagttatggagtgacatatttgaattggttgtttcagaggccaggccagcctccaaagcgcctaatctatctagtgtctgaactggactctggagtccctgacaggttcactggcagtggatcagggacagatttcacactgagaatcagcagagtggaggctgaggatttgggaatttattattgctggcaaggttcacattttcctctcacgttcggtgctgggaccaagctggagctgaaa

SEQ ID NO: 60 - protein, 16 aa, Mus musculus
KSSQGLLDSYGVTYLN

SEQ ID NO: 61 - protein, 7 aa, Mus musculus
LVSELDS

SEQ ID NO: 62 - protein, 9 aa, Mus musculus
WQGSHFPLT

SEQ ID NO: 63 - protein, 122 aa, Mus musculus
EVQLQQSGPELRKPGETVKISCKASGYTFTNYGMNWVKQTPGKGLKWMGWINTYTGERIYADDFKGRFAFSLETSASTAYLQINNLKNEDTATYFCARGEIYYGYDVGFVYWGQGTLVTVSA

SEQ ID NO: 64 - DNA, 366 bp, Mus musculus
gaggtccagttgcagcagtctggacctgagctgaggaagcctggagagacagtcaagatctcctgcaaggcttctgggtataccttcacaaactatggaatgaactgggtgaagcagactccaggaaagggtttaaagtggatgggctggataaacacctacactggagaacgaatatatgctgatgacttcaagggacggtttgccttctctttggaaacctctgccagcactgcctatttgcagatcaacaacctcaaaaatgaggacacggctacatatttctgtgcaagaggggagatctactatggttacgacgtgggctttgtttactggggccaagggactctggtcactgtctctgca

SEQ ID NO: 65 - protein, 6 aa, Mus musculus
TNYGMN

SEQ ID NO: 66 - protein, 17 aa, Mus musculus
WINTYTGERIYADDFKG

SEQ ID NO: 67 - protein, 111 aa, Mus musculus
DIVLTQSPASLVVSLGQRATISCRASKSVSTSGYSYMHWYQQKPGQPPKLLIYLASNLESGVPARFSGSGSGTDFTLNIHPVEEEDAATYYCQHSRELPWTFGGGTRLEIK

SEQ ID NO: 68 - DNA, 333 bp, Mus musculus
gacattgtgctgacacagtctcctgcttccttagttgtatctctggggcagagggccaccatctcatgcagggccagcaaaagtgtcagtacatctggctatagttatatgcactggtaccaacagaaaccaggacagccacccaaactcctcatctatcttgcatccaacctagaatctggggtccctgccaggttcagtggcagtgggtctgggacagacttcaccctcaacatccatcctgtggaggaggaggatgctgcaacctattactgtcagcacagtagggagcttccgtggacgttcggtggaggcaccagactggaaataaaa

SEQ ID NO: 69 - protein, 121 aa, Mus musculus
QVQLQQSGAELVRPGTSVKMSCKAAGYTFTNYWIGWVKQRPGHGLEWIGDIYPGSGDTNYNGKFKGKATLAADISSNAAYMQLSSLTSEDSAIYYCARSYYRNDAASFAYWGQGTLVTVSA

SEQ ID NO: 70 - DNA, 363 bp, Mus musculus
caggtccagctgcagcagtctggagctgagctggtaaggcctgggacttcagtgaagatgtcctgcaaggctgctggatacaccttcactaactactggataggttgggtaaagcagaggcctggacatggccttgagtggattggagatatttaccctggaagtggtgatactaattacaatgggaagttcaagggcaaggccacactggctgcagacatttcctccaacgcagcctacatgcagctcagcagcctgacatctgaggactctgccatctattactgtgcaagaagctactataggaacgacgcggcctcatttgcttactggggccaagggactctggtcactgtctctgca

SEQ ID NO: 71 - protein, 6 aa, Mus musculus
TNYWIG

SEQ ID NO: 72 - protein, 17 aa, Mus musculus
DIYPGSGDTNYNGKFKG

SEQ ID NO: 73 - protein, 12 aa, Mus musculus
SYYRNDAASFAY

SEQ ID NO: 74 - protein, 107 aa, Mus musculus
DIVMTQSHKFMSTSVGDRVNITCKASQDVDTAVAWYQQKPSQSPKLLIYWTSTRHTGVPDRFTGSGSGTDFTLTISNVQSEDLADYFCQQFSSYPLTFGAGTKLELK

SEQ ID NO: 75 - DNA, 321 bp, Mus musculus
gacattgtgatgacccagtctcacaaattcatgtccacatcagtaggagacagggtcaacatcacctgcaaggccagtcaggatgtggatactgctgtagcctggtatcaacagaaaccaagtcaatctcctaaactactgatttactggacatccacccggcacactggagtccctgatcgcttcacaggcagtggatctgggacagatttcactctcaccattagcaatgtgcagtctgaagacttggcagattatttctgtcaacaatttagtagctatcctctcacgttcggtgctgggaccaagctggagctgaaa

SEQ ID NO: 76 - protein, 11 aa, Mus musculus
KASQDVDTAVA

SEQ ID NO: 77 - protein, 7 aa, Mus musculus
WTSTRHT

SEQ ID NO: 78 - protein, 9 aa, Mus musculus
QQFSSYPLT

SEQ ID NO: 79 - protein, 122 aa, Mus musculus
EVQLQQSGPELKKPGETVKISCKASGYIFTNFGMNWVRQAPGKALKWMGWINTYTGEQIYADDFKGRFAFSLETSASTAYLQINNLKNEDTATYFCARGEIYYGYDVGFVYWGQGTLVTVSA

SEQ ID NO: 80 - DNA, 366 bp, Mus musculus
gaggtccagttgcagcagtctggacctgagctgaagaagcctggagagacagtcaagatctcctgcaaggcttctgggtatatcttcacgaactttggaatgaactgggtgaggcaggctccaggaaaggctttaaagtggatgggctggataaacacctacactggagaacaaatatatgctgatgacttcaagggacggtttgccttctctttggaaacctctgccagcactgcctatttgcagatcaacaacctcaaaaatgaggacacggctacatatttctgtgcaagaggggagatctactatggttacgacgtgggctttgtttactggggccaagggactctggtcactgtctctgca

SEQ ID NO: 81 - protein, 111 aa, Mus musculus
DIVLTQSPASLTVSLGQRATISCGASKSVSTSGYSYMHWYQQKPGQPPKLLIYLGSDLESGVPARFSGSGSGTDFTLNIHPVEEEDAATYYCQHSRELPWTFGGGTKLEIK

SEQ ID NO: 82 - DNA, 333 bp, Mus musculus
gacattgtgctgacacagtctcctgcttccttaactgtatctctggggcagagggccaccatctcatgcggggccagcaaaagtgtcagtacatctggctatagttatatgcactggtaccaacagaaaccaggacagccacccaaactcctcatctatcttggatccgacctagaatctggggtccctgccaggttcagtggcagtgggtctgggacagacttcaccctcaacatccatcctgtggaggaggaggatgctgcaacctattactgtcaacacagtagggaacttccgtggacgttcggtggaggcaccaagctggaaatcaaa

SEQ ID NO: 83 - protein, 15 aa, Mus musculus
GASKSVSTSGYSYMH

SEQ ID NO: 84 - protein, 7 aa, Mus musculus
LGSDLES

SEQ ID NO: 85 - protein, 111 aa, Mus musculus
NIVLTQSPASLAVSLGQRATISCRASESVDSSGNSFMHWYQQKPGQPPKLLIYLESNLESGVPARFSGSGSRTDFTLTIEPVEADDAATYYCQQSNEDPWTFGGGTKLEIK

SEQ ID NO: 86 - DNA, 333 bp, Mus musculus
aacattgtgctgacccaatctccagcttctttggctgtgtctctagggcagagggccaccatatcctgcagagccagtgaaagtgttgatagttctggcaatagttttatgcactggtaccagcagaaaccaggacagccacccaaactcctcatctatcttgaatccaacctagaatctggggtccctgccaggttcagtggcagtgggtctaggacagacttcaccctcaccattgaacctgtggaggctgatgatgctgcaacctattactgtcagcaaagtaatgaggatccgtggacgttcggtggaggcaccaagctggaaatcaaa

SEQ ID NO: 87 - protein, 15 aa, Mus musculus
RASESVDSSGNSFMH

SEQ ID NO: 88 - protein, 7 aa, Mus musculus
LESNLES

SEQ ID NO: 89 - protein, 9 aa, Mus musculus
QQSNEDPWT

SEQ ID NO: 90 - protein, 111 aa, Mus musculus
DIVLTQSPASLAISLGQRATISCRASRSVTTSGYSYIHWYQQKPGQPPKLLIYLASDLEAGVPARFSGSGSGTDFTLNIHPVEEEDAATYYCQHSRELPWTFGGGTKLEIK

SEQ ID NO: 91 - DNA, 333 bp, Mus musculus
gacattgtgctgacacagtctcctgcttccttagctatatctctggggcagagggccaccatctcatgcagggccagcagaagtgtcactacatctggctatagttatatacactggtaccaacagaaaccaggacagccacccaaactcctcatctatcttgcatccgacctagaagctggggtccctgccaggttcagtggcagtgggtctgggacagacttcaccctcaacatccatcctgtggaggaagaggatgctgcaacctattactgtcagcacagtagggagcttccgtggacgttcggtggaggcaccaagctggaaataaaa

SEQ ID NO: 92 - protein, 15 aa, Mus musculus
RASRSVTTSGYSYIH

SEQ ID NO: 93 - protein, 109 aa, Homo sapiens
QAVVTQEPSLTVSPGGTVTLTCRSSTGAVTTSNYANWVQQKPGQAPRGLIGGTNKRAPWTPARFSGSLLGGKAALTLSGAQPEDEAEYYCALWYSNLWVFGGGTKLTVL

SEQ ID NO: 94 - DNA, 327 bp, Homo sapiens
caggctgtggtcacacaagagcctagcctgacagtgtctcctggcggcacagtgaccctgacctgtagatcttctacaggcgccgtgaccaccagcaactacgctaattgggtgcagcagaagcccggccaggctcctagaggactgatcggcggaacaaacaagagagccccttggacacccgccagattctctggatctctgctcggcggaaaggccgctctgacactttctggtgctcagcctgaggacgaggccgagtactattgtgccctgtggtacagcaacctgtgggtgttcggcggaggcaccaaactgacagttctg

SEQ ID NO: 95 - protein, 13 aa, Homo sapiens
SSTGAVTTSNYAN

SEQ ID NO: 96 - protein, 8 aa, Homo sapiens
GGTNKRAP

SEQ ID NO: 97 - protein, 9 aa, Homo sapiens
ALWYSNLWV

SEQ ID NO: 98 - protein, 109 aa, Homo sapiens
QAVVTQEPSLTVSPGGTVTLTCRSSTGAVTTSNYANWVQEKPGQAPRGLIGGTNKRAPWTPARFSGSLLGGKAALTLSGAQPEDEAEYYCALWYSNLWVFGGGTKLTVL

SEQ ID NO: 99 - DNA, 327 bp, Homo sapiens
caggctgtggtcacacaagagcctagcctgacagtgtctcctggcggcacagtgaccctgacctgtagatcttctacaggcgccgtgaccaccagcaactacgctaattgggtgcaggagaagcccggccaggctcctagaggactgatcggcggaacaaacaagagagccccttggacacccgccagattctctggatctctgctcggcggaaaggccgctctgacactttctggtgctcagcctgaggacgaggccgagtactattgtgccctgtggtacagcaacctgtgggtgttcggcggaggcaccaaactgacagttctg

SEQ ID NO: 100 - protein, 109 aa, Homo sapiens
EAVVTQEPSLTVSPGGTVTLTCESSDGAVTTSNYANWVQEKPGQAPRGLIGGTNKEAPWTPARFSGSLLGGKAALTLSGAQPEDEAEYYCALWYSNLWVFGGGTKLTVL

SEQ ID NO: 101 - DNA, 327 bp, Homo sapiens
gaggctgtggtcacacaagagcctagcctgacagtgtctcctggcggcacagtgaccctgacctgtgagtcttctgacggcgccgtgaccaccagcaactacgctaattgggtgcaggagaagcccggccaggctcctagaggactgatcggcggaacaaacaaggaggccccttggacacccgccagattctctggatctctgctcggcggaaaggccgctctgacactttctggtgctcagcctgaggacgaggccgagtactattgtgccctgtggtacagcaacctgtgggtgttcggcggaggcaccaaactgacagttctg

SEQ ID NO: 102 - protein, 13 aa, Homo sapiens
SSDGAVTTSNYAN

SEQ ID NO: 103 - protein, 8 aa, Homo sapiens
GGTNKEAP

SEQ ID NO: 104 - protein, 109 aa, Homo sapiens
QAVVTQEPSLTVSPGGTVTLTCESSDGAVTTSNYANWVQEKPGQAPRGLIGGTNKEAPWTPARFSGSLLGGKAALTLSGAQPEDEAEYYCALWYSNLWVFGGGTKLTVL

SEQ ID NO: 105 - DNA, 327 bp, Homo sapiens
caggctgtggtcacacaagagcctagcctgacagtgtctcctggcggcacagtgaccctgacctgtgagtcttctgacggcgccgtgaccaccagcaactacgctaattgggtgcaggagaagcccggccaggctcctagaggactgatcggcggaacaaacaaggaggccccttggacacccgccagattctctggatctctgctcggcggaaaggccgctctgacactttctggtgctcagcctgaggacgaggccgagtactattgtgccctgtggtacagcaacctgtgggtgttcggcggaggcaccaaactgacagttctg

SEQ ID NO: 106 - protein, 109 aa, Homo sapiens
QAVVTQEPSLTVSPGGTVTLTCRSSTGAVTTSNYANWVQEKPGQAPRGLIGGTNKRAPWTPARFSGSLLGGKAALTITGAQAEDEAEYYCVLWYSNLWVFGGGTKLTVL

SEQ ID NO: 107 - DNA, 327 bp, Homo sapiens
caggctgtggtcacacaagagcctagcctgacagtgtctcctggcggcacagtgaccctgacctgtagatcttctacaggcgccgtgaccaccagcaactacgctaattgggtgcaggagaagcccggccaggctcctagaggactgatcggcggaacaaacaagagagccccttggacacccgccagattctctggatctctgctcggcggaaaggccgctctgacaatcactggtgctcaggctgaggacgaggccgagtactattgtgtgctgtggtacagcaacctgtgggtgttcggcggaggcaccaaactgacagttctg

SEQ ID NO: 108 - protein, 9 aa, Homo sapiens
VLWYSNLWV

SEQ ID NO: 109 - protein, 109 aa, Homo sapiens
QAVVTQEPSLTVSPGGTVTLTCRSSTGAVTTSNYANWFQEKPGQAPRGLIYGTNKRAPWTPARFSGSLLGGKAALTLSGAQAEDEAEYYCVLWYSNLWVFGGGTKLTVL

SEQ ID NO: 110 - DNA, 327 bp, Homo sapiens
caggctgtggtcacacaagagcctagcctgacagtgtctcctggcggcacagtgaccctgacctgtagatcttctacaggcgccgtgaccaccagcaactacgctaattggttccaggagaagcccggccaggctcctagaggactgatctacggaacaaacaagagagccccttggacacccgccagattctctggatctctgctcggcggaaaggccgctctgacactttctggtgctcaggctgaggacgaggccgagtactattgtgtcctgtggtacagcaacctgtgggtgttcggcggaggcaccaaactgacagttctg

SEQ ID NO: 111 - protein, 8 aa, Homo sapiens
YGTNKRAP

SEQ ID NO: 112 - protein, 125 aa, Homo sapiens
EVQLVESGGGLVQPGGSLRLSCAASGFTFNTYAMNWVRQAPGKGLEWVSRIRSKYNNYATYYADSVKDRFTISRDDSKNTLYLQMNSLKTEDTAVYYCVRHGNFGNSYVSWFAYWGQGTLVTVSS

SEQ ID NO: 113 - DNA, 375 bp, Homo sapiens
gaggtgcagctggttgaatctggcggaggactggttcagcctggcggatctctgagactgtcttgtgccgccagcggcttcaccttcaacacctacgctatgaactgggtccgacaggcccctggcaaaggactggaatgggtgtccagaatcaggtccaagtacaacaactacgccacctactacgccgacagcgtgaaggacagattcaccatcagcagggacgacagcaagaacaccctgtacctgcagatgaacagcctgagagccgaggacaccgccgtgtactactgtgtcagacacggcaacttcggcaacagctatgtgtcttggtttgcctactggggccagggcacactggtcacagttagctct

SEQ ID NO: 114 - protein, 6 aa, Homo sapiens
NTYAMN

SEQ ID NO: 115 - protein, 18 aa, Homo sapiens
IRSKYNNYATYYADSVKD

SEQ ID NO: 116 - protein, 14 aa, Homo sapiens
HGNFGNSYVSWFAY

SEQ ID NO: 117 - protein, 125 aa, Homo sapiens
EVQLVESGGGLVQPGGSLRLSCAASGFTFSTYAMNWVRKAPGKGLEWVSRIRSKYNNYATYYADSVKDRFTISRDDSKNTLYLQMNSLRAEDTAVYYCVRHGNFGNSYVSWFAYWGQGTLVTVSS

SEQ ID NO: 118 - DNA, 375 bp, Homo sapiens
gaggtgcagctggttgaatctggcggaggactggttcagcctggcggatctctgagactgtcttgtgccgccagcggcttcaccttctccacctacgctatgaactgggtccgaaaggcccctggcaaaggactggaatgggtgtccagaatcaggtccaagtacaacaactacgccacctactacgccgacagcgtgaaggacagattcaccatcagcagggacgacagcaagaacaccctgtacctgcagatgaacagcctgagagccgaggacaccgccgtgtactactgtgtcagacacggcaacttcggcaacagctatgtgtcttggtttgcctactggggccagggcacactggtcacagttagctct

SEQ ID NO: 119 - protein, 6 aa, Homo sapiens
STYAMN

SEQ ID NO: 120 - protein, 125 aa, Homo sapiens
EVQLVESGGGLVQPGGSLRLSCAASGFTFSTYAMNWVRKAPGKGLEWVSRIRSKYNNYATYYADSVKDRFTISRDDSKNTLYLQMNSLRAEDTAVYYCVRHGNFGESYVSWFAYWGQGTLVTVSS

SEQ ID NO: 121 - DNA, 375 bp, Homo sapiens
gaggtgcagctggttgaatctggcggaggactggttcagcctggcggatctctgagactgtcttgtgccgccagcggcttcaccttctccacctacgctatgaactgggtccgaaaggcccctggcaaaggactggaatgggtgtccagaatcaggtccaagtacaacaactacgccacctactacgccgacagcgtgaaggacagattcaccatcagcagggacgacagcaagaacaccctgtacctgcagatgaacagcctgagagccgaggacaccgccgtgtactactgtgtcagacacggcaacttcggcgagagctatgtgtcttggtttgcctactggggccagggcacactggtcacagttagctct

SEQ ID NO: 122 - protein, 14 aa, Homo sapiens
HGNFGESYVSWFAY

SEQ ID NO: 123 - protein, 125 aa, Homo sapiens
EVQLVESGGGLVQPGGSLRLSCAASGFTFSTYAMNWVRKAPGKGLEWVSRIRSKYNNYATYYADSVKDRFTISRDDSKNTLYLQMNSLRAEDTAVYYCVRHGNFGQSYVSWFAYWGQGTLVTVSS

SEQ ID NO: 124 - DNA, 375 bp, Homo sapiens
gaggtgcagctggttgaatctggcggaggactggttcagcctggcggatctctgagactgtcttgtgccgccagcggcttcaccttctccacctacgctatgaactgggtccgaaaggcccctggcaaaggactggaatgggtgtccagaatcaggtccaagtacaacaactacgccacctactacgccgacagcgtgaaggacagattcaccatcagcagggacgacagcaagaacaccctgtacctgcagatgaacagcctgagagccgaggacaccgccgtgtactactgtgtcagacacggcaacttcggccagagctatgtgtcttggtttgcctactggggccagggcacactggtcacagttagctct

SEQ ID NO: 125 - protein, 14 aa, Homo sapiens
HGNFGQSYVSWFAY

SEQ ID NO: 126 - protein, 125 aa, Homo sapiens
EVQLVESGGGLVQPGGSLRLSCAASGFTFSTYAMNWVRKAPGKGLEWVSRIRSKYNNYATYYADSVKDRFTISRDDSKNTLYLQMNSLRAEDTAVYYCVRHGNFGDSYVSWFAYWGQGTLVTVSS

SEQ ID NO: 127 - DNA, 375 bp, Homo sapiens
gaggtgcagctggttgaatctggcggaggactggttcagcctggcggatctctgagactgtcttgtgccgccagcggcttcaccttctccacctacgctatgaactgggtccgaaaggcccctggcaaaggactggaatgggtgtccagaatcaggtccaagtacaacaactacgccacctactacgccgacagcgtgaaggacagattcaccatcagcagggacgacagcaagaacaccctgtacctgcagatgaacagcctgagagccgaggacaccgccgtgtactactgtgtcagacacggcaacttcggcgacagctatgtgtcttggtttgcctactggggccagggcacactggtcacagttagctct

SEQ ID NO: 128 - protein, 14 aa, Homo sapiens
HGNFGDSYVSWFAY

SEQ ID NO: 129 - protein, 125 aa, Homo sapiens
EVQLVESGGGLVQPGGSLRLSCAASGFTFSTYAMNWVRKAPGKGLEWVSRIRSKYNNYATYYADSVKDRFTISRDDSKNTLYLQMNSLRAEDTAVYYCVRHGNFGTSYVSWFAYWGQGTLVTVSS

SEQ ID NO: 130 - DNA, 375 bp, Homo sapiens
gaggtgcagctggttgaatctggcggaggactggttcagcctggcggatctctgagactgtcttgtgccgccagcggcttcaccttctccacctacgctatgaactgggtccgaaaggcccctggcaaaggactggaatgggtgtccagaatcaggtccaagtacaacaactacgccacctactacgccgacagcgtgaaggacagattcaccatcagcagggacgacagcaagaacaccctgtacctgcagatgaacagcctgagagccgaggacaccgccgtgtactactgtgtcagacacggcaacttcggcaccagctatgtgtcttggtttgcctactggggccagggcacactggtcacagttagctct

SEQ ID NO: 131 - protein, 14 aa, Homo sapiens
HGNFGTSYVSWFAY

SEQ ID NO: 132 - protein, 125 aa, Homo sapiens
EVQLVESGGGLVQPGGSLRLSCAASGFTFSDYAMNWVRKAPGKGLEWVSRIRSKYNNYATYYADSVEDRFTISRDDSKNTLYLQMNSLRAEDTAVYYCVRHGNFGNSYVSWFAYWGQGTLVTVSS

SEQ ID NO: 133 - DNA, 375 bp, Homo sapiens
gaggtgcagctggttgaatctggcggaggactggttcagcctggcggatctctgagactgtcttgtgccgccagcggcttcaccttctccgactacgctatgaactgggtccgaaaggcccctggcaaaggactggaatgggtgtccagaatcaggtccaagtacaacaactacgccacctactacgccgacagcgtggaggacagattcaccatcagcagggacgacagcaagaacaccctgtacctgcagatgaacagcctgagagccgaggacaccgccgtgtactactgtgtcagacacggcaacttcggcaacagctatgtgtcttggtttgcctactggggccagggcacactggtcacagttagctct

SEQ ID NO: 134 - protein, 6 aa, Homo sapiens
SDYAMN

SEQ ID NO: 135 - protein, 18 aa, Homo sapiens
IRSKYNNYATYYADSVED

SEQ ID NO: 136 - protein, 125 aa, Homo sapiens
EVQLVESGGGLVQPGGSLRLSCAASGFTFNTYAMNWVRKAPGKGLEWVGRIRSKYNNYATYYADSVKDRFTISRDDSKNSLYLQMNSLKTEDTAVYYCARHGNFGNSYVSWFAYWGQGTLVTVSS

SEQ ID NO: 137 - DNA, 375 bp, Homo sapiens
gaggtgcagctggttgaatctggcggaggactggttcagcctggcggatctctgagactgtcttgtgccgccagcggcttcaccttcaacacctacgctatgaactgggtccgaaaggcccctggcaaaggactggaatgggtgggaagaatcaggtccaagtacaacaactacgccacctactacgccgacagcgtgaaggacagattcaccatcagcagggacgacagcaagaacagcctgtacctgcagatgaacagcctgaaaaccgaggacaccgccgtgtactactgtgccagacacggcaacttcggcaacagctatgtgtcttggtttgcctactggggccagggcacactggtcacagttagctct

SEQ ID NO: 138 - protein, 125 aa, Homo sapiens
EVQLVESGGGLVQPGGSLRLSCAASGFTFNTYAMNWVRKAPGKGLEWVGRIRSKYNNYATYYADSVKDRFTISRDDSKNSLYLQMNSLKTEDTAVYYCVRHGNFGNSYVSWFAYWGQGTLVTVSS

SEQ ID NO: 139 - DNA, 375 bp, Homo sapiens
gaggtgcagctggttgaatctggcggaggactggttcagcctggcggatctctgagactgtcttgtgccgccagcggcttcaccttcaacacctacgctatgaactgggtccgaaaggcccctggcaaaggactggaatgggtgggaagaatcaggtccaagtacaacaactacgccacctactacgccgacagcgtgaaggacagattcaccatcagcagggacgacagcaagaacagcctgtacctgcagatgaacagcctgaaaaccgaggacaccgccgtgtactactgtgtcagacacggcaacttcggcaacagctatgtgtcttggtttgcctactggggccagggcacactggtcacagttagctct

SEQ ID NO: 140 - protein, 125 aa, Homo sapiens
EVQLVESGGGLVQPGGSLRLSCAASGFTFNTYAMNWVRKAPGKGLEWVARIRSKYNNYATYYADSVKDRFTISRDDSKNSLYLQMNSLKTEDTAVYYCVRHGNFGNSYVSWFAYWGQGTLVTVSS

SEQ ID NO: 141 - DNA, 375 bp, Homo sapiens
gaggtgcagctggttgaatctggcggaggactggttcagcctggcggatctctgagactgtcttgtgccgccagcggcttcaccttcaacacctacgctatgaactgggtccgaaaggcccctggcaaaggactggaatgggtggccagaatcaggtccaagtacaacaactacgccacctactacgccgacagcgtgaaggacagattcaccatcagcagggacgacagcaagaacagcctgtacctgcagatgaacagcctgaaaaccgaggacaccgccgtgtactactgtgtcagacacggcaacttcggcaacagctatgtgtcttggtttgcctactggggccagggcacactggtcacagttagctct

SEQ ID NO: 142 - protein, 107 aa, Homo sapiens
DIQMTQSPSSLSASVGDRVTITCQASQDVDTAVAWYQKKPGKAPKLLIYWTSTRHTGVPSRFSGSGSGTDFTFTISSLQPEDIATYFCQQFSSYPLTFGQGTKVEIK

SEQ ID NO: 143 - DNA, 321 bp, Homo sapiens
gacatccagatgacacagagccctagcagcctgtctgccagcgtgggagacagagtgaccatcacctgtcaggccagccaggatgtggatacagccgtggcctggtatcagaagaagcctggcaaggcccctaagctgctgatctactggaccagcaccagacacacaggcgtgccctctagattcagcggctctggctctggcaccgacttcaccttcacaatcagcagcctgcagcctgaggatatcgctacctacttctgccagcagttcagcagctaccctctgacattcggccagggcaccaaggtggaaatcaag

SEQ ID NO: 144 - protein, 11 aa, Homo sapiens
QASQDVDTAVA

SEQ ID NO: 145 - protein, 121 aa, Homo sapiens
QVQLVQSGAEVKKPGSSVKVSCKASGYTFTNYWIGWVREAPGQGLEWMGDIYPGSGDTNYNGKFQGRVTLTADISSNTAYMELSSLRSEDTAVYYCARSYYRNDAASFAYWGQGTLVTVSS

SEQ ID NO: 146 - DNA, 363 bp, Homo sapiens
caggttcagctggttcagtctggcgccgaagtgaagaaacctggcagcagcgtgaaggtgtcctgcaaggctagcggctacacattcaccaactactggatcggctgggtccgagaggctcctggacaaggacttgagtggatgggcgacatctaccctggcagcggcgacacaaactacaacggcaagttccagggcagagtgaccctgacagccgacatcagcagcaacaccgcctacatggaactgagcagcctgagaagcgaggacaccgccgtgtactactgcgccagaagctactacagaaacgacgccgccagcttcgcttactggggacagggaacactggtcaccgtgtctagt

SEQ ID NO: 147 - protein, 17 aa, Homo sapiens
DIYPGSGDTNYNGKFQG

SEQ ID NO: 148 - protein, 111 aa, Homo sapiens
DIVLTQSPASLAVSPGQRATITCRASKSVSTSGYSYMHWYQKKPGQPPKLLIYLASNLESGVPARFSGSGSGTDFTLTINPVEANDTANYYCQHSRELPWTFGQGTKVEIK

SEQ ID NO: 149 - DNA, 333 bp, Homo sapiens
gacatcgtgctgacacagagccctgcttctctggctgtgtctcctggccagagagccaccatcacctgtagagccagcaagagcgtgtccaccagcggctactcttacatgcactggtatcagaagaagcccggccagcctcctaagctgctgatctacctggctagcaacctcgaaagcggagtgcctgctagattttctggcagcggctctggcaccgacttcaccctgacaatcaaccccgtggaagccaacgacaccgccaactactactgccagcacagcagagagctgccctggacatttggccagggcaccaaggtggaaatcaag

SEQ ID NO: 150 - protein, 122 aa, Homo sapiens
QVQLVQSGSELKKPGASVKVSCKASGYTFTNFGMNWVREAPGQGLEWMGWINTYTGDQIYADDFKGRFAFSLDTSASTAYLQISSLKAEDTAVYFCARGEIYYGYDVGFVYWGQGTLVTVSS

SEQ ID NO: 151 - DNA, 366 bp, Homo sapiens
caggttcagctggtgcagtctggcagcgagctgaagaaacctggcgcctctgtgaaggtgtcctgcaaggctagcggctacacattcaccaacttcggcatgaactgggtccgagaggctcctggacagggactcgaatggatgggctggatcaacacctacaccggcgaccagatctacgccgacgacttcaagggcagattcgccttcagcctggacacctctgccagcacagcttacctgcagatcagcagcctgaaggccgaggataccgccgtgtacttctgtgccagaggcgagatctactacggctacgatgtgggcttcgtctactggggacagggaacactggtcaccgttagctct

SEQ ID NO: 152 - protein, 111 aa, Homo sapiens
DIVLTQSPASLAVSPGQRATITCRASRSVTTSGYSYIHWYQKKPGQPPKLLIYLASDLEAGVPARFSGSGSGTDFTLTINPVEANDTANYYCQHSRELPWTFGQGTKVEIK

SEQ ID NO: 153 - DNA, 333 bp, Homo sapiens
gacatcgtgctgacacagagccctgcttctctggctgtgtctcctggccagagagccaccatcacctgtagagccagcagaagcgtgaccaccagcggctactcttacatccactggtatcagaagaagcccggccagcctcctaagctgctgatctacctggccagcgatctggaagctggcgtgccagctagattttctggcagcggctctggcaccgacttcaccctgacaatcaaccccgtggaagccaacgacaccgccaactactactgccagcacagcagagagctgccctggacatttggccagggcaccaaggtggaaatcaag

SEQ ID NO: 154 - protein, 122 aa, Homo sapiens
QVQLVQSGSELKKPGASVKVSCKASGYIFTNFGMNWVREAPGQGLEWMGWINTYTGEQIYADDFKGRFAFSLDTSASTAYLQISSLKAEDTAVYFCARGEIYYGYDVGFVYWGQGTLVTVSS

SEQ ID NO: 155 - DNA, 366 bp, Homo sapiens
caggttcagctggtgcagtctggcagcgagctgaagaaacctggcgcctctgtgaaggtgtcctgcaaggctagcggctacatcttcaccaacttcggcatgaactgggtccgagaggctcctggacagggactcgaatggatgggctggatcaacacctacaccggcgagcagatctacgccgatgacttcaaaggcagattcgcgttcagcctggacaccagcgccagcacagcttacctgcagatcagctctctgaaggccgaggataccgccgtgtacttctgtgccagaggcgagatctactacggctacgacgtgggctttgtgtactggggccagggaacactggtcaccgttagctct

SEQ ID NO: 156 - protein, 111 aa, Homo sapiens
DIVLTQSPASLAVSPGQRATITCRASKSVSTSGYSYMHWYQKKPGQPPKLLIYLGSDLESGVPARFSGSGSGTDFTLTINPVEANDTANYYCQHSRELPWTFGQGTKVEIK

SEQ ID NO: 157 - DNA, 333 bp, Homo sapiens
gacatcgtgctgacacagagccctgcttctctggctgtgtctcctggccagagagccaccatcacctgtagagccagcaagagcgtgtccaccagcggctactcttacatgcactggtatcagaagaagcccggccagcctcctaagctgctgatctacctgggtagcgacctcgaaagcggagtgcctgctagattttctggcagcggctctggcaccgacttcaccctgacaatcaaccccgtggaagccaacgacaccgccaactactactgccagcacagcagagagctgccctggacatttggccagggcaccaaggtggaaatcaag

SEQ ID NO: 158 - protein, 122 aa, Homo sapiens; identical to SEQ ID NO: 154

SEQ ID NO: 159 - DNA, 366 bp, Homo sapiens; identical to SEQ ID NO: 155

SEQ ID NO: 160 - protein, 111 aa, Homo sapiens; identical to SEQ ID NO: 148

SEQ ID NO: 161 - DNA, 333 bp, Homo sapiens; identical to SEQ ID NO: 149

SEQ ID NO: 162 - protein, 122 aa, Homo sapiens; identical to SEQ ID NO: 154

SEQ ID NO: 163 - DNA, 366 bp, Homo sapiens; identical to SEQ ID NO: 155

SEQ ID NO: 164 - protein, 111 aa, Homo sapiens; identical to SEQ ID NO: 148

SEQ ID NO: 165 - DNA, 333 bp, Homo sapiens; identical to SEQ ID NO: 149

SEQ ID NO: 166 - protein, 122 aa, Homo sapiens
QVQLVQSGSELKKPGASVKVSCKASGYTFTNFGMNWVREAPGQGLEWMGWINTYTGDLIYGDDFKGRFAFSLDTSASTAYLQISSLKAEDTAVYFCARGEIYYGYDVGFAYWGQGTLVTVSS

SEQ ID NO: 167 - DNA, 366 bp, Homo sapiens
caggttcagctggtgcagtctggcagcgagctgaagaaacctggcgcctctgtgaaggtgtcctgcaaggctagcggctacacattcaccaacttcggcatgaactgggtccgagaggctcctggacagggactcgaatggatgggctggatcaacacctacaccggcgacctgatctacggcgacgacttcaagggcagattcgccttcagcctggacacctctgccagcacagcttacctgcagatcagcagcctgaaggccgaggataccgccgtgtacttctgtgccagaggcgagatctactacggctacgatgtgggcttcgcctactggggacagggaacactggtcaccgttagctct

SEQ ID NO: 168 - protein, 111 aa, Homo sapiens; identical to SEQ ID NO: 148

SEQ ID NO: 169 - DNA, 333 bp, Homo sapiens; identical to SEQ ID NO: 149

SEQ ID NO: 170 - protein, 122 aa, Homo sapiens
QVQLVQSGSELKKPGASVKVSCKASGYTFTNYGMNWVREAPGQGLEWMGWINTYTGERIYADDFKGRFAFSLDTSASTAYLQISSLKAEDTAVYFCARGEIYYGYDVGFVYWGQGTLVTVSS

SEQ ID NO: 171 - DNA, 366 bp, Homo sapiens
caggttcagctggtgcagtctggcagcgagctgaagaaacctggcgcctctgtgaaggtgtcctgcaaggctagcggctacacattcaccaactacggcatgaactgggtccgagaggctcctggacagggactcgaatggatgggctggatcaacacctacaccggcgaaaggatctacgccgacgacttcaagggcagattcgccttcagcctggacacctctgccagcacagcttacctgcagatcagcagcctgaaggccgaggataccgccgtgtacttctgtgccagaggcgagatctactacggctacgatgtgggcttcgtctactggggacagggaacactggtcaccgttagctct

SEQ ID NO: 172 - protein, 218 aa, Homo sapiens
DIVLTQSPASLAVSPGQRATITCRASKSVSTSGYSYMHWYQKKPGQPPKLLIYLASNLESGVPARFSGSGSGTDFTLTINPVEAEDTANYYCQHSRELPWTFGQGTKVEIKRTVAAPSVFIFPPSDEQLKSGTASVVCLLNNFYPREAKVQWKVDNALQSGNSQESVTEQDSKDSTYSLSSTLTLSKADYEKHKVYACEVTHQGLSSPVTKSFNRGEC

SEQ ID NO: 173 - DNA, 654 bp, Homo sapiens
gacatcgtgctgacacagagccctgcttctctggctgtgtctcctggccagagagccaccatcacctgtagagccagcaagagcgtgtccaccagcggctactcttacatgcactggtatcagaagaagcccggccagcctcctaagctgctgatctacctggctagcaacctcgaaagcggagtgcctgctagattttctggcagcggctctggcaccgacttcaccctgacaatcaaccccgtggaagccgaagacaccgccaactactactgccagcacagcagagagctgccctggacatttggccagggcaccaaggtggaaatcaagcgaactgtggctgcaccatctgtcttcatcttcccgccatctgatgagcagttgaaatctggaactgcctctgttgtgtgcctgctgaataacttctatcccagagaggccaaagtacagtggaaggtggataacgccctccaatcgggtaactcccaggagagtgtcacagagcaggacagcaaggacagcacctacagcctcagcagcaccctgacgctgagcaaagcagactacgagaaacacaaagtctacgcctgcgaagtcacccatcagggcctgagctcgcccgtcacaaagagcttcaacaggggagagtgt

SEQ ID NO: 174 - protein, 449 aa, Homo sapiens
QVQLVQSGSELKKPGASVKVSCKASGYIFTNFGMNWVREAPGQGLEWMGWINTYTGEQIYADGFTGRFVFSLDTSASTAYLQISSLKAEDTAVYFCARGEIYYGYDVGFVYWGQGTLVTVSSASTKGPSVFPLAPCSRSTSESTAALGCLVKDYFPEPVTVSWNSGALTSGVHTFPAVLQSSGLYSLSSVVTVPSSSLGTKTYTCNVDHKPSNTKVDKRVESKYGPPCPPCPAPEFEGGPSVFLFPPKPKDTLMISRTPEVTCVVVDVSQEDPEVQFNWYVDGVEVHNAKTKPREEQFNSTYRVVSVLTVLHQDWLNGKEYKCKVSNKGLASSIEKTISKAKGQPREPQVCTLPPSQEEMTKNQVSLSCAVKGFYPSDIAVEWESNGQPENNYKTTPPVLDSDGSFFLVSKLTVDKSRWQEGNVFSCSVMHEALHNHYTQKSLSLSLGK

SEQ ID NO: 175 - DNA, 1347 bp, Homo sapiens
caggttcagctggtgcagtctggcagcgagctgaagaaacctggcgcctctgtgaaggtgtcctgcaaggctagcggctacatcttcaccaacttcggcatgaactgggtccgagaggctcctggacagggactcgaatggatgggctggatcaacacctacaccggcgagcagatctacgccgatggcttcacaggcagattcgtgttcagcctggacaccagcgccagcacagcttacctgcagatcagctctctgaaggccgaggataccgccgtgtacttctgtgccagaggcgagatctactacggctacgacgtgggctttgtgtactggggccagggaacactggtcaccgttagctctgctagcaccaagggccccagcgtgttccccctggccccttgcagcagaagcaccagcgagagcacagccgccctgggctgcctggtgaaggactacttccccgagcccgtgaccgtgtcctggaacagcggcgctctgaccagcggcgtgcataccttccccgccgtgctccagagcagcggactgtactccctgagcagcgtggtgaccgtgccttccagcagcctgggcaccaagacctacacctgcaacgtggaccacaagcccagcaacaccaaggtggacaagagagtggagagcaagtacggccctccctgccccccttgccctgcccccgagttcgagggcggacctagcgtgttcctgttcccccccaagcccaaggacaccctgatgatcagcagaacccccgaggtgacctgcgtggtggtggacgtgtcccaggaggaccccgaggtccagtttaattggtacgtggacggcgtggaagtgcataacgccaagaccaagcccagagaggagcagttcaacagcacctacagagtggtgtccgtgctgaccgtgctgcaccaggactggctgaacggcaaggaatacaagtgcaaggtctccaacaagggcctggccagcagcatcgagaagaccatcagcaaggccaagggccagccacgggagccccaggtctgcaccctgccacctagccaagaggagatgaccaagaaccaggtgtccctgagctgtgccgtgaaaggcttctatcccagcgatatcgccgtggagtgggagagcaacggccagcccgagaacaactacaagaccaccccccctgtgctggacagcgacggcagcttcttcctggtttccaagctgaccgtggacaagtccagatggcaggagggcaacgtcttcagctgctccgtgatgcacgaggccctgcacaaccactacacccagaagtccctgagcctgagcctgggcaag

SEQ ID NO: 176 - protein, 218 aa, Homo sapiens
DIVLTQSPASLAVSPGQRATITCRASKSVTTSGYSYIHWYQKKPGQPPKLLIYLASDLEAGVPARFSGSGSGTDFTLTINPVEAEDTANYYCQHSRELPWTFGQGTKVEIKRTVAAPSVFIFPPSDEQLKSGTASVVCLLNNFYPREAKVQWKVDNALQSGNSQESVTEQDSKDSTYSLSSTLTLSKADYEKHKVYACEVTHQGLSSPVTKSFNRGEC

SEQ ID NO: 177 - DNA, 654 bp, Homo sapiens
gacatcgtgctgacacagagccctgcttctctggctgtgtctcctggccagagagccaccatcacctgtagagccagcaagagcgtgaccaccagcggctactcttacatccactggtatcagaagaagcccggccagcctcctaagctgctgatctacctggccagcgatctggaagctggcgtgccagctagattttctggcagcggctctggcaccgacttcaccctgacaatcaaccccgtggaagccgaagacaccgccaactactactgccagcacagcagagagctgccctggacatttggccagggcaccaaggtggaaatcaagcgaactgtggctgcaccatctgtcttcatcttcccgccatctgatgagcagttgaaatctggaactgcctctgttgtgtgcctgctgaataacttctatcccagagaggccaaagtacagtggaaggtggataacgccctccaatcgggtaactcccaggagagtgtcacagagcaggacagcaaggacagcacctacagcctcagcagcaccctgacgctgagcaaagcagactacgagaaacacaaagtctacgcctgcgaagtcacccatcagggcctgagctcgcccgtcacaaagagcttcaacaggggagagtgt

SEQ ID NO: 178 - protein, 449 aa, Homo sapiens
QVQLVQSGSELKKPGASVKVSCKASGYIFTNFGMNWVREAPGQGLEWMGWINTYTGEQIYADGFTGRFVFSLDTSVSTAYLQISSLKAEDTAVYFCARGEIYYGYDVGFVYWGQGTLVTVSSASTKGPSVFPLAPCSRSTSESTAALGCLVKDYFPEPVTVSWNSGALTSGVHTFPAVLQSSGLYSLSSVVTVPSSSLGTKTYTCNVDHKPSNTKVDKRVESKYGPPCPPCPAPEFEGGPSVFLFPPKPKDTLMISRTPEVTCVVVDVSQEDPEVQFNWYVDGVEVHNAKTKPREEQFNSTYRVVSVLTVLHQDWLNGKEYKCKVSNKGLASSIEKTISKAKGQPREPQVCTLPPSQEEMTKNQVSLSCAVKGFYPSDIAVEWESNGQPENNYKTTPPVLDSDGSFFLVSKLTVDKSRWQEGNVFSCSVMHEALHNHYTQKSLSLSLGK

SEQ ID NO: 179 - DNA, 1347 bp, Homo sapiens
caggttcagctggtgcagtctggcagcgagctgaagaaacctggcgcctctgtgaaggtgtcctgcaaggctagcggctacatcttcaccaacttcggcatgaactgggtccgagaggctcctggacagggactcgaatggatgggctggatcaacacctacaccggcgagcagatctacgccgatggcttcacaggcagattcgtgttcagcctggacaccagcgtcagcacagcttacctgcagatcagctctctgaaggccgaggataccgccgtgtacttctgtgccagaggcgagatctactacggctacgacgtgggctttgtgtactggggccagggaacactggtcaccgttagctctgctagcaccaagggccccagcgtgttccccctggccccttgcagcagaagcaccagcgagagcacagccgccctgggctgcctggtgaaggactacttccccgagcccgtgaccgtgtcctggaacagcggcgctctgaccagcggcgtgcataccttccccgccgtgctccagagcagcggactgtactccctgagcagcgtggtgaccgtgccttccagcagcctgggcaccaagacctacacctgcaacgtggaccacaagcccagcaacaccaaggtggacaagagagtggagagcaagtacggccctccctgccccccttgccctgcccccgagttcgagggcggacctagcgtgttcctgttcccccccaagcccaaggacaccctgatgatcagcagaacccccgaggtgacctgcgtggtggtggacgtgtcccaggaggaccccgaggtccagtttaattggtacgtggacggcgtggaagtgcataacgccaagaccaagcccagagaggagcagttcaacagcacctacagagtggtgtccgtgctgaccgtgctgcaccaggactggctgaacggcaaggaatacaagtgcaaggtctccaacaagggcctggccagcagcatcgagaagaccatcagcaaggccaagggccagccacgggagccccaggtctgcaccctgccacctagccaagaggagatgaccaagaaccaggtgtccctgagctgtgccgtgaaaggcttctatcccagcgatatcgccgtggagtgggagagcaacggccagcccgagaacaactacaagaccaccccccctgtgctggacagcgacggcagcttcttcctggtttccaagctgaccgtggacaagtccagatggcaggagggcaacgtcttcagctgctccgtgatgcacgaggccctgcacaaccactacacccagaagtccctgagcctgagcctgggcaag

SEQ ID NO: 180 - protein, 215 aa, Homo sapiens
QAVVTQEPSLTVSPGGTVTLTCRSSTGAVTTSNYANWVQEKPGQAPRGLIGGTNKRAPWTPARFSGSLLGGKAALTITGAQAEDEAEYYCVLWYSNLWVFGGGTKLTVLGQPKAAPSVTLFPPSSEELQANKATLVCLISDFYPGAVTVAWKADSSPVKAGVETTTPSKQSNNKYAASSYLSLTPEQWKSHRSYSCQVTHEGSTVEKTVAPTECS

SEQ ID NO: 181 - DNA, 645 bp, Homo sapiens
caggctgtggtcacacaagagcctagcctgacagtgtctcctggcggcacagtgaccctgacctgtagatcttctacaggcgccgtgaccaccagcaactacgctaattgggtgcaggagaagcccggccaggctcctagaggactgatcggcggaacaaacaagagagccccttggacacccgccagattctctggatctctgctcggcggaaaggccgctctgacaatcactggtgctcaggctgaggacgaggccgagtactattgtgtgctgtggtacagcaacctgtgggtgttcggcggaggcaccaaactgacagttctgggtcagcccaaggcggcgccctcggtcactctgttcccgccctcctctgaggagcttcaagccaacaaggccacactggtgtgtctcataagtgacttctatccgggagccgtgacagtggcctggaaggcagatagcagccccgtcaaggcgggagtggagaccaccacaccctccaaacaaagcaacaacaagtacgcggccagcagctacctgagcctgacgcctgagcagtggaagtcccacagaagctacagctgccaggtcacgcatgaagggagcaccgtggagaagacagtggcccctacagaatgttca

SEQ ID NO: 182 - protein, 452 aa, Homo sapiens
EVQLVESGGGLVQPGGSLRLSCAASGFTFNTYAMNWVRKAPGKGLEWVGRIRSKYNNYATYYADSVKDRFTISRDDSKNSLYLQMNSLKTEDTAVYYCVRHGNFGNSYVSWFAYWGQGTLVTVSSASTKGPSVFPLAPCSRSTSESTAALGCLVKDYFPEPVTVSWNSGALTSGVHTFPAVLQSSGLYSLSSVVTVPSSSLGTKTYTCNVDHKPSNTKVDKRVESKYGPPCPPCPAPEFEGGPSVFLFPPKPKDTLMISRTPEVTCVVVDVSQEDPEVQFNWYVDGVEVHNAKTKPREEQFNSTYRVVSVLTVLHQDWLNGKEYKCKVSNKGLASSIEKTISKAKGQPREPQVYTLPPCQEEMTKNQVSLWCLVKGFYPSDIAVEWESNGQPENNYKTTPPVLDSDGSFFLYSKLTVDKSRWQEGNVFSCSVMHEALHNHYTQKSLSLSLGK

SEQ ID NO: 183 - DNA, 1356 bp, Homo sapiens
gaggtgcagctggttgaatctggcggaggactggttcagcctggcggatctctgagactgtcttgtgccgccagcggcttcaccttcaacacctacgctatgaactgggtccgaaaggcccctggcaaaggactggaatgggtgggaagaatcaggtccaagtacaacaactacgccacctactacgccgacagcgtgaaggacagattcaccatcagcagggacgacagcaagaacagcctgtacctgcagatgaacagcctgaaaaccgaggacaccgccgtgtactactgtgtcagacacggcaacttcggcaacagctatgtgtcttggtttgcctactggggccagggcacactggtcacagttagctctgctagcaccaagggccccagcgtgttccccctggccccttgcagcagaagcaccagcgagagcacagccgccctgggctgcctggtgaaggactacttccccgagcccgtgaccgtgtcctggaacagcggcgctctgaccagcggcgtgcataccttccccgccgtgctccagagcagcggactgtactccctgagcagcgtggtgaccgtgccttccagcagcctgggcaccaagacctacacctgcaacgtggaccacaagcccagcaacaccaaggtggacaagagagtggagagcaagtacggccctccctgccccccttgccctgcccccgagttcgagggcggacctagcgtgttcctgttcccccccaagcccaaggacaccctgatgatcagcagaacccccgaggtgacctgcgtggtggtggacgtgtcccaggaggaccccgaggtccagtttaattggtacgtggacggcgtggaagtgcataacgccaagaccaagcccagagaggagcagttcaacagcacctacagagtggtgtccgtgctgaccgtgctgcaccaggactggctgaacggcaaggaatacaagtgcaaggtctccaacaagggcctggccagcagcatcgagaagaccatcagcaaggccaagggccagccacgggagccccaggtctacaccctgccaccttgtcaagaggagatgaccaagaaccaggtgtccctgtggtgtctggtgaaaggcttctatcccagcgatatcgccgtggagtgggagagcaacggccagcccgagaacaactacaagaccaccccccctgtgctggacagcgacggcagcttcttcctgtactccaagctgaccgtggacaagtccagatggcaggagggcaacgtcttcagctgctccgtgatgcacgaggccctgcacaaccactacacccagaagtccctgagcctgagcctgggcaag

SEQ ID NO: 184 - protein, 109 aa, Mus musculus
QAVVTQESALTTSPGETVTLTCRSSTGAVTTSNYANWVQQKPDHLFTGLIGGTNKRAPGVPARFSGSLIGDKAALTITGAQTEDEAIYFCALWYSNLWVFGGGTKLTVL

SEQ ID NO: 185 - protein, 125 aa, Mus musculus
EVQLVESGGGLVQPKGSLKLSCAASGFTFNTYAMNWVRQAPGKGLEWVARIRSKYNNYATYYADSVKDRFTISRDDSQSILYLQMNNLKTEDTAMYYCVRHGNFGNSYVSWFAYWGQGTLVTVSS